European Patent Application EP 4 653 005 A1, published November 26, 2025. Title: 毛螺菌科微生物菌株、预防或治疗肿瘤的药物及应用. Applicant: 慕恩（广州）生物科技有限公司. The sequence listing filed with the application follows.

SEQUENCE LISTING (3 sequences)

SEQ ID NO: 1 - DNA, 1383 bp, synthetic construct
  source 1..1383: mol_type = other DNA
cagtcgagcgagcattttaaaggaagttttcggatggaatttgaaatgactgagcggcggacgggtgagtaacgcgtgggtaacctgcctcatacagggggataacagttagaaatgactgctaataccgcataagcacacagtaccgcatggtacggtgtgaaaaactccggtggtatgagatggacccgcgtctgattagctggttggcggggtaacggcccaccaaggcgacgatcagtagccgacctgagagggtgaccggccacattgggactgagacacggcccaaactcctacgggaggcagcagtggggaatattgcacaatgggggaaaccctgatgcagcaacgccgcgtgagtgaagaagtatttcggtatgtaaagctctatcagcagggaagaaagtgacggtacctgactaagaagccccggctaactacgtgccagcagccgcggtaatacgtagggggcaagcgttatccggatttactgggtgtaaagggagcgtagacggcacagcaagtctgaagtgaaatccccgggctcaacccgggaactgctttggaaactgttgggctggagtgctggagaggcaagcggaattcctagtgtagcggtgaaatgcgtagatattaggaggaacaccagtggcgaaggcggcttgctggacagtaactgacgttgaggctcgaaagcgtggggagcaaacaggattagataccctggtagtccacgccgtaaacgatgcatactaggtgtcggggagcaaagcttttccgtggccgcccaaacgcagtaagtatgccacctggggagtacgttcgcaagaatgaaactcaaaggaattgacggggacccgcacaagcggtggagcatgtggtttaattcgaagcaacgcgaagaaccttaccaagtcttgacatccccctgacgagcaagtaacgttgcttttccttcgggacaggggagacaggtggtgcatggttgtcgtcagctcgtgtcgtgagatgttgggttaagtcccgcaacgagcgcaacccttattgtcagtagccagcaggtaaagctgggcactctgatgagactgccagggataacctggaggaaggtggggatgacgtcaaatcatcatgccccttatgatttgggctacacacgtgctacaatggcgtaaacaaagggaagcgaccctgcgaaggcaagcaaatcccaaaaataacgtcccagttcggattgtagtctgcaactcgactacatgaagctggaatcgctagtaatcgcagatcagcatgctgcggtgaatacgttcccgggtcttgtacacaccgcccgtcacaccatgggagtcggaaatgcccgaagccagtgacccaactgca

SEQ ID NO: 2 - DNA, 20 bp, synthetic construct
  source 1..20: mol_type = other DNA
agagtttgatcmtggctcag

SEQ ID NO: 3 - DNA, 22 bp, synthetic construct
  source 1..22: mol_type = other DNA
tacggytaccttgttacgactt